European Patent Specification EP 3 814 527 B1, published February 22, 2023. Title: CRISPR Effector System Based Amplification Methods, Systems, and Diagnostics. Applicant: The Broad Institute, Inc. Massachusetts Institute of Technology President and Fellows of Harvard College Zhang, Feng Kellner, Max Gootenberg, Jonathan Abudayyeh, Omar. The sequence listing filed with the application follows.

SEQUENCE LISTING (24 sequences)

SEQ ID NO: 1 - protein, 44 aa, Escherichia coli
  misc_feature (27)..(27): Xaa can be any naturally occurring amino acid
TKFYDRKEIKDILAYLRLIANPDDDSXKRIINVPKRGIGAATVD

SEQ ID NO: 2 - protein, 44 aa, Escherichia coli
TKFYDRKEIKDILAYLRLVSNPDDDSFARIVNVPKRGIGATSVD

SEQ ID NO: 3 - protein, 44 aa, Escherichia coli
TKFYDRKEIKDLLAYLRLIANPADDSLQRIINVPKRGLGSTSLD

SEQ ID NO: 4 - protein, 45 aa, Escherichia coli
HRFYDRMEVKDIIAYLRVIQDPEGDLSIKRIINVPKRGIGKATID

SEQ ID NO: 5 - protein, 45 aa, Escherichia coli
LRFYERKEIKDIVAYLRFISNPADAVSFRRVVNVPKRGIGDATVQ

SEQ ID NO: 6 - protein, 45 aa, Escherichia coli
LKFYQRKEIKDIMAYLRVVANPSDDVSLLRIINVPRRGIGEATVY

SEQ ID NO: 7 - protein, 44 aa, Escherichia coli
LRFYDRKEIKDLIAYLRILVNPYDDSFKRIINVPKRGIGAATIE

SEQ ID NO: 8 - protein, 44 aa, Escherichia coli
TKFYERKEIKDLVAYLRVLQNVQDDSLKRIINVPKRGIGLRTIE

SEQ ID NO: 9 - protein, 44 aa, Escherichia coli
IKFYDRKEIKDLLAYLRLIANQDDDSLARIVNVPKRGVGATSVD

SEQ ID NO: 10 - protein, 45 aa, Escherichia coli
HKFYDRKEIKDLLAYLNIINNPRDGVSFERVVNTPKRGIGAASVE

SEQ ID NO: 11 - protein, 45 aa, Escherichia coli
TKFYDRKEIKDLLAYLRLIANNDDDLSLARIINEPKRSIGATSFE

SEQ ID NO: 12 - protein, 44 aa, Escherichia coli
TKFYDRKEIKDLLAYLRLIANPDDDSLRRVINVPKRGIGATSMD

SEQ ID NO: 13 - protein, 44 aa, Escherichia coli
LREYDRKEIKDILAYLRLIVNPYDDSFKRIVNVPRRGIGPATIE

SEQ ID NO: 14 - protein, 45 aa, Escherichia coli
MRFFERQEIKDALSYLRLIANRNDDAAFERVVNTPTRGIGDRTLD

SEQ ID NO: 15 - protein, 6 aa, Artificial Sequence
  Synthetic Peptide
  misc (2)..(2): Xaa = asparagine, histidine, or lysine
  misc (3)..(3): Xaa = arginine, serine, aspartic acid, glutamic acid, glutamine, asparagine, glycine, tyrosine, or histidine
  misc (4)..(4): Xaa = isoleucine, serine, threonine, valine, or leucine
  misc (5)..(5): Xaa = leucine, phenylalanine, asparagine, tyrosine, valine, isoleucine, serine, aspartic acid, glutamic acid, or alanine
RXXXXH

SEQ ID NO: 16 - protein, 6 aa, Artificial Sequence
  Synthetic Peptide
  MISC_FEATURE (2)..(2): Xaa = asparagine or histidine
  MISC_FEATURE (3)..(3): Xaa = arginine, serine, aspartic acid, glutamic acid, glutamine, asparagine, glycine, tyrosine, or histidine
  MISC_FEATURE (4)..(4): Xaa = isoleucine, serine, threonine, valine, or leucine
  MISC_FEATURE (5)..(5): Xaa = leucine, phenylalanine, asparagine, tyrosine, valine, isoleucine, serine, aspartic acid, glutamic acid, or alanine
RXXXXH

SEQ ID NO: 17 - protein, 6 aa, Artificial Sequence
  Synthetic Peptide
  MISC_FEATURE (2)..(2): Xaa = asparagine or lysine
  MISC_FEATURE (3)..(3): Xaa = arginine, serine, aspartic acid, glutamic acid, glutamine, asparagine, glycine, tyrosine, or histidine
  MISC_FEATURE (4)..(4): Xaa = isoleucine, serine, threonine, valine, or leucine
  MISC_FEATURE (5)..(5): Xaa = leucine, phenylalanine, asparagine, tyrosine, valine, isoleucine, serine, aspartic acid, glutamic acid, or alanine
RXXXXH

SEQ ID NO: 18 - RNA, 25 nt, Artificial Sequence
  Synthetic Oligonucleotide
gggaacaaagcugaaguacuuaccc

SEQ ID NO: 19 - DNA, 18 bp, Artificial Sequence
  Synthetic Oligonucleotide
gggtagggcgggttggga

SEQ ID NO: 20 - DNA, 25 bp, Artificial Sequence
  Synthetic Oligonucleotide
  misc_feature (25)..(25): 3' ThioMC3-D modification
ttataactattcctaaaaaaaaaaa

SEQ ID NO: 21 - DNA, 26 bp, Artificial Sequence
  Synthetic Oligonucleotide
  misc_feature (1)..(1): 5' ThioMC6-D modification
aaaaaaaaaactcccctaataacaat

SEQ ID NO: 22 - RNA, 45 nt, Artificial Sequence
  Synthetic Oligonucleotide
ggguaggaauaguuauaauuucccuuucccauuguuauuagggag

SEQ ID NO: 23 - RNA, 12 nt, Artificial Sequence
  Synthetic Oligonucleotide
  misc_feature (1)..(1): 5' Biosg modification
  misc_feature (12)..(12): 3' IAbRQSp modification
ucucguacguuc

SEQ ID NO: 24 - RNA, 24 nt, Artificial Sequence
  Synthetic Oligonucleotide
  misc_feature (1)..(1): 5' Biosg modification
  misc_feature (24)..(24): 3' IAbRQSp modification
ucucguacguucucucguacguuc